European Patent Specification EP 3 452 102 B1, published June 12, 2024. Title: GENE THERAPY FOR TREATING HEMOPHILIA A. Applicant: The Trustees of the University of Pennsylvania. The sequence listing filed with the application follows.

SEQUENCE LISTING (20 sequences)

SEQ ID NO: 1 - DNA, 4371 bp, Homo sapiens
atgcaaatagagctctccacctgcttctttctgtgccttttgcgattctgctttagtgccaccagaagatactacctgggtgcagtggaactgtcatgggactatatgcaaagtgatctcggtgagctgcctgtggacgcaagatttcctcctagagtgccaaaatcttttccattcaacacctcagtcgtgtacaaaaagactctgtttgtagaattcacggatcaccttttcaacatcgctaagccaaggccaccctggatgggtctgctaggtcctaccatccaggctgaggtttatgatacagtggtcattacacttaagaacatggcttcccatcctgtcagtcttcatgctgttggtgtatcctactggaaagcttctgagggagctgaatatgatgatcagaccagtcaaagggagaaagaagatgataaagtcttccctggtggaagccatacatatgtctggcaggtcctgaaagagaatggtccaatggcctctgacccactgtgccttacctactcatatctttctcatgtggacctggtaaaagacttgaattcaggcctcattggagccctactagtatgtagagaagggagtctggccaaggaaaagacacagaccttgcacaaatttatactactttttgctgtatttgatgaagggaaaagttggcactcagaaacaaagaactccttgatgcaggatagggatgctgcatctgctcgggcctggcctaaaatgcacacagtcaatggttatgtaaacaggtctctgccaggtctgattggatgccacaggaaatcagtctattggcatgtgattggaatgggcaccactcctgaagtgcactcaatattcctcgaaggtcacacatttcttgtgaggaaccatcgccaggcgtccttggaaatctcgccaataactttccttactgctcaaacactcttgatggaccttggacagtttctactgttttgtcatatctcttcccaccaacatgatggcatggaagcttatgtcaaagtagacagctgtccagaggaaccccaactacgaatgaaaaataatgaagaagcggaagactatgatgatgatcttactgattctgaaatggatgtggtcaggtttgatgatgacaactctccttcctttatccaaattcgctcagttgccaagaagcatcctaaaacttgggtacattacattgctgctgaagaggaggactgggactatgctcccttagtcctcgcccccgatgacagaagttataaaagtcaatatttgaacaatggccctcagcggattggtaggaagtacaaaaaagtccgatttatggcatacacagatgaaacctttaagactcgtgaagctattcagcatgaatcaggaatcttgggacctttactttatggggaagttggagacacactgttgattatatttaagaatcaagcaagcagaccatataacatctaccctcacggaatcactgatgtccgtcctttgtattcaaggagattaccaaaaggtgtaaaacatttgaaggattttccaattctgccaggagaaatattcaaatataaatggacagtgactgtagaagatgggccaactaaatcagatcctcggtgcctgacccgctattactctagtttcgttaatatggagagagatctagcttcaggactcattggccctctcctcatctgctacaaagaatctgtagatcaaagaggaaaccagataatgtcagacaagaggaatgtcatcctgttttctgtatttgatgagaaccgaagctggtacctcacagagaatatacaacgctttctccccaatccagctggagtgcagcttgaggatccagagttccaagcctccaacatcatgcacagcatcaatggctatgtttttgatagtttgcagttgtcagtttgtttgcatgaggtggcatactggtacattctaagcattggagcacagactgacttcctttctgtcttcttctctggatataccttcaaacacaaaatggtctatgaagacacactcaccctattcccattctcaggagaaactgtcttcatgtcgatggaaaacccaggtctatggattctggggtgccacaactcagactttcggaacagaggcatgaccgccttactgaaggtttctagttgtgacaagaacactggtgattattacgaggacagttatgaagatatttcagcatacttgctgagtaaaaacaatgccattgaaccaagaagcttctcccagaatccaccagtcttgaaacgccatcaacgggaaataactcgtactactcttcagtcagatcaagaggaaattgactatgatgataccatatcagttgaaatgaagaaggaagattttgacatttatgatgaggatgaaaatcagagcccccgcagctttcaaaagaaaacacgacactattttattgctgcagtggagaggctctgggattatgggatgagtagctccccacatgttctaagaaacagggctcagagtggcagtgtccctcagttcaagaaagttgttttccaggaatttactgatggctcctttactcagcccttataccgtggagaactaaatgaacatttgggactcctggggccatatataagagcagaagttgaagataatatcatggtaactttcagaaatcaggcctctcgtccctattccttctattctagccttatttcttatgaggaagatcagaggcaaggagcagaacctagaaaaaactttgtcaagcctaatgaaaccaaaacttacttttggaaagtgcaacatcatatggcacccactaaagatgagtttgactgcaaagcctgggcttatttctctgatgttgacctggaaaaagatgtgcactcaggcctgattggaccccttctggtctgccacactaacacactgaaccctgctcatgggagacaagtgacagtacaggaatttgctctgtttttcaccatctttgatgagaccaaaagctggtacttcactgaaaatatggaaagaaactgcagggctccctgcaatatccagatggaagatcccacttttaaagagaattatcgcttccatgcaatcaatggctacataatggatacactacctggcttagtaatggctcaggatcaaaggattcgatggtatctgctcagcatgggcagcaatgaaaacatccattctattcatttcagtggacatgtgttcactgtacgaaaaaaagaggagtataaaatggcactgtacaatctctatccaggtgtttttgagacagtggaaatgttaccatccaaagctggaatttggcgggtggaatgccttattggcgagcatctacatgctgggatgagcacactttttctggtgtacagcaataagtgtcagactcccctgggaatggcttctggacacattagagattttcagattacagcttcaggacaatatggacagtgggccccaaagctggccagacttcattattccggatcaatcaatgcctggagcaccaaggagcccttttcttggatcaaggtggatctgttggcaccaatgattattcacggcatcaagacccagggtgcccgtcagaagttctccagcctctacatctctcagtttatcatcatgtatagtcttgatgggaagaagtggcagacttatcgaggaaattccactggaaccttaatggtcttctttggcaatgtggattcatctgggataaaacacaatatttttaaccctccaattattgctcgatacatccgtttgcacccaactcattatagcattcgcagcactcttcgcatggagttgatgggctgtgatttaaatagttgcagcatgccattgggaatggagagtaaagcaatatcagatgcacagattactgcttcatcctactttaccaatatgtttgccacctggtctccttcaaaagctcgacttcacctccaagggaggagtaatgcctggagacctcaggtgaataatccaaaagagtggctgcaagtggacttccagaagacaatgaaagtcacaggagtaactactcagggagtaaaatctctgcttaccagcatgtatgtgaaggagttcctcatctccagcagtcaagatggccatcagtggactctcttttttcagaatggcaaagtaaaggtttttcagggaaatcaagactccttcacacctgtggtgaactctctagacccaccgttactgactcgctaccttcgaattcacccccagagttgggtgcaccagattgccctgaggatggaggttctgggctgcgaggcacaggacctctac

SEQ ID NO: 2 - DNA, 4374 bp, Artificial Sequence
  constructed sequence
atgcagatcgagctgagcacctgcttcttcctgtgcctgctgcggttctgcttctccgccacccggcggtactacctgggagccgtggagctgagctgggattacatgcagagcgatctgggagagctgccagtggatgcccggttcccaccacgggtgccaaagagcttcccattcaacaccagcgtggtgtacaagaagaccctgttcgtggagttcaccgatcacctgttcaacatcgccaagccacggccaccctggatgggactgctgggaccaaccatccaggccgaggtgtacgataccgtggtgatcaccctgaagaacatggcctctcatcctgtgtccctgcacgccgtgggagtgagctactggaaggccagcgagggagccgagtacgatgatcagaccagccagcgggagaaggaggatgataaggtgttcccaggaggaagccacacctacgtgtggcaggtgctgaaggagaacggaccaatggccagcgatccactgtgcctgacctacagctacctgagccacgtggatctggtgaaggatctgaacagcggactgatcggagccctgctggtgtgccgggagggaagcctggccaaggagaagacccagaccctgcacaagttcatcctgctgttcgccgtgttcgatgagggaaagagctggcacagcgagaccaagaacagcctgatgcaggatcgggatgccgccagcgcccgggcctggccaaagatgcacaccgtgaacggatacgtgaaccggagcctgccaggactgatcggatgccaccggaagagcgtgtactggcacgtgatcggaatgggaaccaccccagaggtgcactctatcttcctggagggacacacctttctggtgcggaaccaccggcaggccagcctggagatcagcccaatcaccttcctgaccgcccagaccctgctgatggatctgggacagttcctgctgttctgccatatcagcagccaccagcacgatggaatggaggcctacgtgaaggtggatagctgcccagaggagccacagctgcggatgaagaacaacgaggaggccgaggattacgatgatgatctgaccgatagcgagatggatgtggtgcggttcgatgatgataacagcccaagcttcatccagatccggagcgtggccaagaagcacccaaagacctgggtgcactacatcgccgccgaggaggaggattgggattacgccccactggtgctggcccctgatgatcggagctacaagagccagtacctgaacaacggaccacagcggatcggacggaagtacaaaaaagtgcggttcatggcctacaccgatgagaccttcaagacccgggaggccatccagcacgagagcggaatcctgggaccactgctgtacggagaggtgggagataccctgctgatcatcttcaagaaccaggccagccggccatacaacatctacccacacggaatcaccgatgtgcggccactgtacagccggcggctgccaaagggagtgaagcacctgaaggatttcccaatcctgccaggagagatcttcaagtacaagtggacagtgacagtggaggatggaccaaccaagtctgatccaagatgcctgaccagatactacagcagctttgtgaacatggagagagacctggcctctggactgattggaccactgctgatctgctacaaggagtctgtggatcagagaggaaaccagatcatgtctgataagagaaatgtgatcctgttctctgtgtttgatgagaacagaagctggtacctgacagagaacatccagagattcctgccaaacccagccggagtgcagctggaggatccagagttccaggccagcaacatcatgcacagcatcaacggatacgtgttcgatagcctgcagctgagcgtgtgcctgcacgaggtggcctattggtatatcctgagcatcggagcccagaccgatttcctgagcgtgttcttcagcggatacaccttcaagcacaagatggtgtacgaggataccctgaccctgttcccattctccggagagaccgtgttcatgagcatggagaacccaggactgtggatcctgggatgccacaactctgatttcagaaacagaggaatgactgccctgctgaaagtgtccagctgtgataagaacactggagattactatgaggatagctatgaggatatctctgcctacctgctgagcaagaacaatgccattgagccaagaagcttcagccagaacccaccagtgctgaagagacaccagagagagatcaccagaaccaccctgcagtctgatcaggaggagattgattatgatgataccatctctgtggagatgaagaaggaggattttgatatctatgatgaggatgagaaccagagcccaagaagcttccagaagaagaccagacactacttcatcgctgcagtggagagactgtgggattatggaatgagcagcagcccacacgtgctgagaaacagagcccagagcggatctgtgccacagttcaagaaggtggtgttccaggagttcaccgatggaagcttcacccagccactgtaccggggagagctgaacgagcacctgggactgctgggaccatacatccgggccgaggtggaggataacatcatggtgaccttccggaaccaggccagccggccatacagcttctacagcagcctgatcagctacgaggaggatcagcggcagggagccgagccacggaagaacttcgtgaagccaaacgagaccaagacctacttctggaaggtgcagcaccacatggccccaaccaaggatgagttcgattgcaaggcctgggcctacttcagcgatgtggatctggagaaggatgtgcacagcggactgatcggaccactgctggtgtgccacaccaacaccctgaacccagcccacggacggcaggtgaccgtgcaggagttcgccctgttcttcaccatcttcgatgagaccaagagctggtacttcaccgagaacatggagcggaactgccgggccccttgcaacatccagatggaggatccaaccttcaaggagaactaccggttccacgccatcaacggatacatcatggataccctgccaggactggtgatggcccaggatcagcggatccggtggtacctgctgagcatgggaagcaacgagaacatccacagcatccacttcagcggacacgtgttcaccgtgcggaagaaggaggagtacaagatggccctgtacaacctgtacccaggagtgttcgagaccgtggagatgctgccaagcaaggccggaatctggcgggtggagtgcctgatcggagagcacctgcacgccggaatgagcaccctgttcctggtgtacagcaacaagtgccagaccccactgggaatggccagcggacacatccgggatttccagatcaccgccagcggacagtacggacagtgggccccaaagctggcccggctgcactacagcggaagcatcaacgcctggagcaccaaggagccattcagctggatcaaagtggatctgctggccccaatgatcatccacggaatcaagacccagggagcccggcagaagttcagcagcctgtacatcagccagttcatcatcatgtacagcctggatggaaagaagtggcagacctaccggggaaacagcaccggaaccctgatggtgttcttcggaaacgtggatagcagcggaatcaagcacaacatcttcaacccaccaatcatcgcccgatacatccggctgcacccaacccactacagcatcagaagcaccctgcggatggagctgatgggatgtgatctgaacagctgctccatgccactgggaatggagagcaaggccatcagcgatgcccagatcaccgccagcagctacttcaccaacatgttcgccacctggagcccaagcaaggcccggctgcacctgcagggacggagcaacgcctggcggccacaggtgaataacccaaaggagtggctgcaggtggatttccagaagaccatgaaggtgaccggagtgaccacccagggagtgaagagcctgctgactagcatgtatgtgaaggagttcctgatcagcagcagccaggatggacaccagtggaccctgttcttccagaacggaaaggtgaaggtgttccagggaaaccaggatagcttcaccccagtggtgaacagcctggatccaccactgctgacccgatacctgcggatccacccacagagctgggtgcaccagatcgccctgagaatggaggtgctgggatgcgaggcccaggatctgtactga

SEQ ID NO: 3 - protein, 1457 aa, Homo sapiens
MQIELSTCFFLCLLRFCFSATRRYYLGAVELSWDYMQSDLGELPVDARFPPRVPKSFPFNTSVVYKKTLFVEFTDHLFNIAKPRPPWMGLLGPTIQAEVYDTVVITLKNMASHPVSLHAVGVSYWKASEGAEYDDQTSQREKEDDKVFPGGSHTYVWQVLKENGPMASDPLCLTYSYLSHVDLVKDLNSGLIGALLVCREGSLAKEKTQTLHKFILLFAVFDEGKSWHSETKNSLMQDRDAASARAWPKMHTVNGYVNRSLPGLIGCHRKSVYWHVIGMGTTPEVHSIFLEGHTFLVRNHRQASLEISPITFLTAQTLLMDLGQFLLFCHISSHQHDGMEAYVKVDSCPEEPQLRMKNNEEAEDYDDDLTDSEMDVVRFDDDNSPSFIQIRSVAKKHPKTWVHYIAAEEEDWDYAPLVLAPDDRSYKSQYLNNGPQRIGRKYKKVRFMAYTDETFKTREAIQHESGILGPLLYGEVGDTLLIIFKNQASRPYNIYPHGITDVRPLYSRRLPKGVKHLKDFPILPGEIFKYKWTVTVEDGPTKSDPRCLTRYYSSFVNMERDLASGLIGPLLICYKESVDQRGNQIMSDKRNVILFSVFDENRSWYLTENIQRFLPNPAGVQLEDPEFQASNIMHSINGYVFDSLQLSVCLHEVAYWYILSIGAQTDFLSVFFSGYTFKHKMVYEDTLTLFPFSGETVFMSMENPGLWILGCHNSDFRNRGMTALLKVSSCDKNTGDYYEDSYEDISAYLLSKNNAIEPRSFSQNPPVLKRHQREITRTTLQSDQEEIDYDDTISVEMKKEDFDIYDEDENQSPRSFQKKTRHYFIAAVERLWDYGMSSSPHVLRNRAQSGSVPQFKKVVFQEFTDGSFTQPLYRGELNEHLGLLGPYIRAEVEDNIMVTFRNQASRPYSFYSSLISYEEDQRQGAEPRKNFVKPNETKTYFWKVQHHMAPTKDEFDCKAWAYFSDVDLEKDVHSGLIGPLLVCHTNTLNPAHGRQVTVQEFALFFTIFDETKSWYFTENMERNCRAPCNIQMEDPTFKENYRFHAINGYIMDTLPGLVMAQDQRIRWYLLSMGSNENIHSIHFSGHVFTVRKKEEYKMALYNLYPGVFETVEMLPSKAGIWRVECLIGEHLHAGMSTLFLVYSNKCQTPLGMASGHIRDFQITASGQYGQWAPKLARLHYSGSINAWSTKEPFSWIKVDLLAPMIIHGIKTQGARQKFSSLYISQFIIMYSLDGKKWQTYRGNSTGTLMVFFGNVDSSGIKHNIFNPPIIARYIRLHPTHYSIRSTLRMELMGCDLNSCSMPLGMESKAISDAQITASSYFTNMFATWSPSKARLHLQGRSNAWRPQVNNPKEWLQVDFQKTMKVTGVTTQGVKSLLTSMYVKEFLISSSQDGHQWTLFFQNGKVKVFQGNQDSFTPVVNSLDPPLLTRYLRIHPQSWVHQIALRMEVLGCEAQDLY

SEQ ID NO: 4 - DNA, 34 bp, Artificial Sequence
  constructed sequence
tgtttgctgcttgcaatgtttgcccattttaggg

SEQ ID NO: 5 - DNA, 100 bp, Artificial Sequence
  constructed sequence
ctacctcgtgatcgcccggcccctgttcaaacatgtcctaatactctgtctctgcaagggtcatcagtagttttccatcttactcaacatcctcccagtg

SEQ ID NO: 6 - DNA, 42 bp, Artificial Sequence
  constructed sequence
aggttaatttttaaactgtttgctctggttaataatctcagg

SEQ ID NO: 7 - DNA, 190 bp, Artificial Sequence
  constructed sequence
atttcatagaacgaatgttccgatgctctaatctctctagacaaggttcatatttgtatgggttacttattctctctttgttgactaagtcaataatcagaatcagcaggtttgcagtcagattggcagggataagcagcctagctcaggagaagtgagtataaaagccccaggctgggagcagccatca

SEQ ID NO: 8 - DNA, 176 bp, Artificial Sequence
  constructed sequence
actcaaagttcaaaccttatcattttttgctttgttcctcttggccttggttttgtacatcagctttgaaaataccatcccagggttaatgctggggttaatttataactaagagtgctctagttttgcaatacaggacatgctataaaaatggaaagatgttgctttctgagaga

SEQ ID NO: 9 - DNA, 218 bp, Artificial Sequence
  constructed sequence
tggacacaggacgctgtggtttctgagccagggggcgactcagatcccagccagtggacttagcccctgtttgctcctccgataactggggtgaccttggttaatattcaccagcagcctcccccgttgcccctctggatccactgcttaaatacggacgaggacagggccctgtctcctcagcttcaggcaccaccactgacctgggacagtgaata

SEQ ID NO: 10 - DNA, 75 bp, Artificial Sequence
  constructed sequence
aataaagtctgagtgggcggcagcctgtgtgtgcctgggttctctctgtcccggaatgtgcaaacaatggaggtg

SEQ ID NO: 11 - DNA, 168 bp, Artificial Sequence
  constructed sequence
ctgcgcgctcgctcgctcactgaggccgcccgggcaaagcccgggcgtcgggcgacctttggtcgcccggcctcagtgagcgagcgagcgcgcagagagggagtggccaactccatcactaggggttccttgtagttaatgattaacccgccatgctacttatctact

SEQ ID NO: 12 - DNA, 164 bp, Artificial Sequence
  constructed sequence
gataagtagcatggcgggttaatcattaactacaaggaacccctagtgatggagttggccactccctctctgcgcgctcgctcgctcactgaggccgggcgaccaaaggtcgcccgacgcccgggctttgcccgggcggcctcagtgagcgagcgagcgcgcag

SEQ ID NO: 13 - DNA, 7920 bp, Artificial Sequence
  constructed sequence
ctgcgcgctcgctcgctcactgaggccgcccgggcaaagcccgggcgtcgggcgacctttggtcgcccggcctcagtgagcgagcgagcgcgcagagagggagtggccaactccatcactaggggttccttgtagttaatgattaacccgccatgctacttatctacttaagctacctcgtgatcgcccggcccctgttcaaacatgtcctaatactctgtctctgcaagggtcatcagtagttttccatcttactcaacatcctcccagtggaattcatttcatagaacgaatgttccgatgctctaatctctctagacaaggttcatatttgtatgggttacttattctctctttgttgactaagtcaataatcagaatcagcaggtttgcagtcagattggcagggataagcagcctagctcaggagaagtgagtataaaagccccaggctgggagcagccatcagcggccgccaccatgcagatcgagctgagcacctgcttcttcctgtgcctgctgcggttctgcttctccgccacccggcggtactacctgggagccgtggagctgagctgggattacatgcagagcgatctgggagagctgccagtggatgcccggttcccaccacgggtgccaaagagcttcccattcaacaccagcgtggtgtacaagaagaccctgttcgtggagttcaccgatcacctgttcaacatcgccaagccacggccaccctggatgggactgctgggaccaaccatccaggccgaggtgtacgataccgtggtgatcaccctgaagaacatggcctctcatcctgtgtccctgcacgccgtgggagtgagctactggaaggccagcgagggagccgagtacgatgatcagaccagccagcgggagaaggaggatgataaggtgttcccaggaggaagccacacctacgtgtggcaggtgctgaaggagaacggaccaatggccagcgatccactgtgcctgacctacagctacctgagccacgtggatctggtgaaggatctgaacagcggactgatcggagccctgctggtgtgccgggagggaagcctggccaaggagaagacccagaccctgcacaagttcatcctgctgttcgccgtgttcgatgagggaaagagctggcacagcgagaccaagaacagcctgatgcaggatcgggatgccgccagcgcccgggcctggccaaagatgcacaccgtgaacggatacgtgaaccggagcctgccaggactgatcggatgccaccggaagagcgtgtactggcacgtgatcggaatgggaaccaccccagaggtgcactctatcttcctggagggacacacctttctggtgcggaaccaccggcaggccagcctggagatcagcccaatcaccttcctgaccgcccagaccctgctgatggatctgggacagttcctgctgttctgccatatcagcagccaccagcacgatggaatggaggcctacgtgaaggtggatagctgcccagaggagccacagctgcggatgaagaacaacgaggaggccgaggattacgatgatgatctgaccgatagcgagatggatgtggtgcggttcgatgatgataacagcccaagcttcatccagatccggagcgtggccaagaagcacccaaagacctgggtgcactacatcgccgccgaggaggaggattgggattacgccccactggtgctggcccctgatgatcggagctacaagagccagtacctgaacaacggaccacagcggatcggacggaagtacaaaaaagtgcggttcatggcctacaccgatgagaccttcaagacccgggaggccatccagcacgagagcggaatcctgggaccactgctgtacggagaggtgggagataccctgctgatcatcttcaagaaccaggccagccggccatacaacatctacccacacggaatcaccgatgtgcggccactgtacagccggcggctgccaaagggagtgaagcacctgaaggatttcccaatcctgccaggagagatcttcaagtacaagtggacagtgacagtggaggatggaccaaccaagtctgatccaagatgcctgaccagatactacagcagctttgtgaacatggagagagacctggcctctggactgattggaccactgctgatctgctacaaggagtctgtggatcagagaggaaaccagatcatgtctgataagagaaatgtgatcctgttctctgtgtttgatgagaacagaagctggtacctgacagagaacatccagagattcctgccaaacccagccggagtgcagctggaggatccagagttccaggccagcaacatcatgcacagcatcaacggatacgtgttcgatagcctgcagctgagcgtgtgcctgcacgaggtggcctattggtatatcctgagcatcggagcccagaccgatttcctgagcgtgttcttcagcggatacaccttcaagcacaagatggtgtacgaggataccctgaccctgttcccattctccggagagaccgtgttcatgagcatggagaacccaggactgtggatcctgggatgccacaactctgatttcagaaacagaggaatgactgccctgctgaaagtgtccagctgtgataagaacactggagattactatgaggatagctatgaggatatctctgcctacctgctgagcaagaacaatgccattgagccaagaagcttcagccagaacccaccagtgctgaagagacaccagagagagatcaccagaaccaccctgcagtctgatcaggaggagattgattatgatgataccatctctgtggagatgaagaaggaggattttgatatctatgatgaggatgagaaccagagcccaagaagcttccagaagaagaccagacactacttcatcgctgcagtggagagactgtgggattatggaatgagcagcagcccacacgtgctgagaaacagagcccagagcggatctgtgccacagttcaagaaggtggtgttccaggagttcaccgatggaagcttcacccagccactgtaccggggagagctgaacgagcacctgggactgctgggaccatacatccgggccgaggtggaggataacatcatggtgaccttccggaaccaggccagccggccatacagcttctacagcagcctgatcagctacgaggaggatcagcggcagggagccgagccacggaagaacttcgtgaagccaaacgagaccaagacctacttctggaaggtgcagcaccacatggccccaaccaaggatgagttcgattgcaaggcctgggcctacttcagcgatgtggatctggagaaggatgtgcacagcggactgatcggaccactgctggtgtgccacaccaacaccctgaacccagcccacggacggcaggtgaccgtgcaggagttcgccctgttcttcaccatcttcgatgagaccaagagctggtacttcaccgagaacatggagcggaactgccgggccccttgcaacatccagatggaggatccaaccttcaaggagaactaccggttccacgccatcaacggatacatcatggataccctgccaggactggtgatggcccaggatcagcggatccggtggtacctgctgagcatgggaagcaacgagaacatccacagcatccacttcagcggacacgtgttcaccgtgcggaagaaggaggagtacaagatggccctgtacaacctgtacccaggagtgttcgagaccgtggagatgctgccaagcaaggccggaatctggcgggtggagtgcctgatcggagagcacctgcacgccggaatgagcaccctgttcctggtgtacagcaacaagtgccagaccccactgggaatggccagcggacacatccgggatttccagatcaccgccagcggacagtacggacagtgggccccaaagctggcccggctgcactacagcggaagcatcaacgcctggagcaccaaggagccattcagctggatcaaagtggatctgctggccccaatgatcatccacggaatcaagacccagggagcccggcagaagttcagcagcctgtacatcagccagttcatcatcatgtacagcctggatggaaagaagtggcagacctaccggggaaacagcaccggaaccctgatggtgttcttcggaaacgtggatagcagcggaatcaagcacaacatcttcaacccaccaatcatcgcccgatacatccggctgcacccaacccactacagcatcagaagcaccctgcggatggagctgatgggatgtgatctgaacagctgctccatgccactgggaatggagagcaaggccatcagcgatgcccagatcaccgccagcagctacttcaccaacatgttcgccacctggagcccaagcaaggcccggctgcacctgcagggacggagcaacgcctggcggccacaggtgaataacccaaaggagtggctgcaggtggatttccagaagaccatgaaggtgaccggagtgaccacccagggagtgaagagcctgctgactagcatgtatgtgaaggagttcctgatcagcagcagccaggatggacaccagtggaccctgttcttccagaacggaaaggtgaaggtgttccagggaaaccaggatagcttcaccccagtggtgaacagcctggatccaccactgctgacccgatacctgcggatccacccacagagctgggtgcaccagatcgccctgagaatggaggtgctgggatgcgaggcccaggatctgtactgatgagcatgcaataaagtctgagtgggcggcagcctgtgtgtgcctgggttctctctgtcccggaatgtgcaaacaatggaggtgctcgagtagataagtagcatggcgggttaatcattaactacaaggaacccctagtgatggagttggccactccctctctgcgcgctcgctcgctcactgaggccgggcgaccaaaggtcgcccgacgcccgggctttgcccgggcggcctcagtgagcgagcgagcgcgcagccttaattaacctaattcactggccgtcgttttacaacgtcgtgactgggaaaaccctggcgttacccaacttaatcgccttgcagcacatccccctttcgccagctggcgtaatagcgaagaggcccgcaccgatcgcccttcccaacagttgcgcagcctgaatggcgaatgggacgcgccctgtagcggcgcattaagcgcggcgggtgtggtggttacgcgcagcgtgaccgctacacttgccagcgccctagcgcccgctcctttcgctttcttcccttcctttctcgccacgttcgccggctttccccgtcaagctctaaatcgggggctccctttagggttccgatttagtgctttacggcacctcgaccccaaaaaacttgattagggtgatggttcacgtagtgggccatcgccctgatagacggtttttcgccctttgacgttggagtccacgttctttaatagtggactcttgttccaaactggaacaacactcaaccctatctcggtctattcttttgatttataagggattttgccgatttcggcctattggttaaaaaatgagctgatttaacaaaaatttaacgcgaattttaacaaaatattaacgcttacaatttaggtggcacttttcggggaaatgtgcgcggaacccctatttgtttatttttctaaatacattcaaatatgtatccgctcatgagacaataaccctgataaatgcttcaataatattgaaaaaggaagagtatgagtattcaacatttccgtgtcgcccttattcccttttttgcggcattttgccttcctgtttttgctcacccagaaacgctggtgaaagtaaaagatgctgaagatcagttgggtgcacgagtgggttacatcgaactggatctcaacagcggtaagatccttgagagttttcgccccgaagaacgttttccaatgatgagcacttttaaagttctgctatgtggcgcggtattatcccgtattgacgccgggcaagagcaactcggtcgccgcatacactattctcagaatgacttggttgagtactcaccagtcacagaaaagcatcttacggatggcatgacagtaagagaattatgcagtgctgccataaccatgagtgataacactgcggccaacttacttctgacaacgatcggaggaccgaaggagctaaccgcttttttgcacaacatgggggatcatgtaactcgccttgatcgttgggaaccggagctgaatgaagccataccaaacgacgagcgtgacaccacgatgcctgtagcaatggcaacaacgttgcgcaaactattaactggcgaactacttactctagcttcccggcaacaattaatagactggatggaggcggataaagttgcaggaccacttctgcgctcggcccttccggctggctggtttattgctgataaatctggagccggtgagcgtgggtctcgcggtatcattgcagcactggggccagatggtaagccctcccgtatcgtagttatctacacgacggggagtcaggcaactatggatgaacgaaatagacagatcgctgagataggtgcctcactgattaagcattggtaactgtcagaccaagtttactcatatatactttagattgatttaaaacttcatttttaatttaaaaggatctaggtgaagatcctttttgataatctcatgaccaaaatcccttaacgtgagttttcgttccactgagcgtcagaccccgtagaaaagatcaaaggatcttcttgagatcctttttttctgcgcgtaatctgctgcttgcaaacaaaaaaaccaccgctaccagcggtggtttgtttgccggatcaagagctaccaactctttttccgaaggtaactggcttcagcagagcgcagataccaaatactgttcttctagtgtagccgtagttaggccaccacttcaagaactctgtagcaccgcctacatacctcgctctgctaatcctgttaccagtggctgctgccagtggcgataagtcgtgtcttaccgggttggactcaagacgatagttaccggataaggcgcagcggtcgggctgaacggggggttcgtgcacacagcccagcttggagcgaacgacctacaccgaactgagatacctacagcgtgagctatgagaaagcgccacgcttcccgaagggagaaaggcggacaggtatccggtaagcggcagggtcggaacaggagagcgcacgagggagcttccagggggaaacgcctggtatctttatagtcctgtcgggtttcgccacctctgacttgagcgtcgatttttgtgatgctcgtcaggggggcggagcctatggaaaaacgccagcaacgcggcctttttacggttcctggccttttgctggccttttgctcacatgttctttcctgcgttatcccctgattctgtggataaccgtattaccgcctttgagtgagctgataccgctcgccgcagccgaacgaccgagcgcagcgagtcagtgagcgaggaagcggaagagcgcccaatacgcaaaccgcctctccccgcgcgttggccgattcattaatgcagctggcacgacaggtttcccgactggaaagcgggcagtgagcgcaacgcaattaatgtgagttagctcactcattaggcaccccaggctttacactttatgcttccggctcgtatgttgtgtggaattgtgagcggataacaatttcacacaggaaacagctatgaccatgattacgccagatttaattaagg

SEQ ID NO: 14 - DNA, 8004 bp, Artificial Sequence
  constructed sequence
ctgcgcgctcgctcgctcactgaggccgcccgggcaaagcccgggcgtcgggcgacctttggtcgcccggcctcagtgagcgagcgagcgcgcagagagggagtggccaactccatcactaggggttccttgtagttaatgattaacccgccatgctacttatctacttaagctacctcgtgatcgcccggcccctgttcaaacatgtcctaatactctgtctctgcaagggtcatcagtagttttccatcttactcaacatcctcccagtgaggttaatttttaaactgtttgctctggttaataatctcaggaggttaatttttaaactgtttgctctggttaataatctcagggaattcatttcatagaacgaatgttccgatgctctaatctctctagacaaggttcatatttgtatgggttacttattctctctttgttgactaagtcaataatcagaatcagcaggtttgcagtcagattggcagggataagcagcctagctcaggagaagtgagtataaaagccccaggctgggagcagccatcagcggccgccaccatgcagatcgagctgagcacctgcttcttcctgtgcctgctgcggttctgcttctccgccacccggcggtactacctgggagccgtggagctgagctgggattacatgcagagcgatctgggagagctgccagtggatgcccggttcccaccacgggtgccaaagagcttcccattcaacaccagcgtggtgtacaagaagaccctgttcgtggagttcaccgatcacctgttcaacatcgccaagccacggccaccctggatgggactgctgggaccaaccatccaggccgaggtgtacgataccgtggtgatcaccctgaagaacatggcctctcatcctgtgtccctgcacgccgtgggagtgagctactggaaggccagcgagggagccgagtacgatgatcagaccagccagcgggagaaggaggatgataaggtgttcccaggaggaagccacacctacgtgtggcaggtgctgaaggagaacggaccaatggccagcgatccactgtgcctgacctacagctacctgagccacgtggatctggtgaaggatctgaacagcggactgatcggagccctgctggtgtgccgggagggaagcctggccaaggagaagacccagaccctgcacaagttcatcctgctgttcgccgtgttcgatgagggaaagagctggcacagcgagaccaagaacagcctgatgcaggatcgggatgccgccagcgcccgggcctggccaaagatgcacaccgtgaacggatacgtgaaccggagcctgccaggactgatcggatgccaccggaagagcgtgtactggcacgtgatcggaatgggaaccaccccagaggtgcactctatcttcctggagggacacacctttctggtgcggaaccaccggcaggccagcctggagatcagcccaatcaccttcctgaccgcccagaccctgctgatggatctgggacagttcctgctgttctgccatatcagcagccaccagcacgatggaatggaggcctacgtgaaggtggatagctgcccagaggagccacagctgcggatgaagaacaacgaggaggccgaggattacgatgatgatctgaccgatagcgagatggatgtggtgcggttcgatgatgataacagcccaagcttcatccagatccggagcgtggccaagaagcacccaaagacctgggtgcactacatcgccgccgaggaggaggattgggattacgccccactggtgctggcccctgatgatcggagctacaagagccagtacctgaacaacggaccacagcggatcggacggaagtacaaaaaagtgcggttcatggcctacaccgatgagaccttcaagacccgggaggccatccagcacgagagcggaatcctgggaccactgctgtacggagaggtgggagataccctgctgatcatcttcaagaaccaggccagccggccatacaacatctacccacacggaatcaccgatgtgcggccactgtacagccggcggctgccaaagggagtgaagcacctgaaggatttcccaatcctgccaggagagatcttcaagtacaagtggacagtgacagtggaggatggaccaaccaagtctgatccaagatgcctgaccagatactacagcagctttgtgaacatggagagagacctggcctctggactgattggaccactgctgatctgctacaaggagtctgtggatcagagaggaaaccagatcatgtctgataagagaaatgtgatcctgttctctgtgtttgatgagaacagaagctggtacctgacagagaacatccagagattcctgccaaacccagccggagtgcagctggaggatccagagttccaggccagcaacatcatgcacagcatcaacggatacgtgttcgatagcctgcagctgagcgtgtgcctgcacgaggtggcctattggtatatcctgagcatcggagcccagaccgatttcctgagcgtgttcttcagcggatacaccttcaagcacaagatggtgtacgaggataccctgaccctgttcccattctccggagagaccgtgttcatgagcatggagaacccaggactgtggatcctgggatgccacaactctgatttcagaaacagaggaatgactgccctgctgaaagtgtccagctgtgataagaacactggagattactatgaggatagctatgaggatatctctgcctacctgctgagcaagaacaatgccattgagccaagaagcttcagccagaacccaccagtgctgaagagacaccagagagagatcaccagaaccaccctgcagtctgatcaggaggagattgattatgatgataccatctctgtggagatgaagaaggaggattttgatatctatgatgaggatgagaaccagagcccaagaagcttccagaagaagaccagacactacttcatcgctgcagtggagagactgtgggattatggaatgagcagcagcccacacgtgctgagaaacagagcccagagcggatctgtgccacagttcaagaaggtggtgttccaggagttcaccgatggaagcttcacccagccactgtaccggggagagctgaacgagcacctgggactgctgggaccatacatccgggccgaggtggaggataacatcatggtgaccttccggaaccaggccagccggccatacagcttctacagcagcctgatcagctacgaggaggatcagcggcagggagccgagccacggaagaacttcgtgaagccaaacgagaccaagacctacttctggaaggtgcagcaccacatggccccaaccaaggatgagttcgattgcaaggcctgggcctacttcagcgatgtggatctggagaaggatgtgcacagcggactgatcggaccactgctggtgtgccacaccaacaccctgaacccagcccacggacggcaggtgaccgtgcaggagttcgccctgttcttcaccatcttcgatgagaccaagagctggtacttcaccgagaacatggagcggaactgccgggccccttgcaacatccagatggaggatccaaccttcaaggagaactaccggttccacgccatcaacggatacatcatggataccctgccaggactggtgatggcccaggatcagcggatccggtggtacctgctgagcatgggaagcaacgagaacatccacagcatccacttcagcggacacgtgttcaccgtgcggaagaaggaggagtacaagatggccctgtacaacctgtacccaggagtgttcgagaccgtggagatgctgccaagcaaggccggaatctggcgggtggagtgcctgatcggagagcacctgcacgccggaatgagcaccctgttcctggtgtacagcaacaagtgccagaccccactgggaatggccagcggacacatccgggatttccagatcaccgccagcggacagtacggacagtgggccccaaagctggcccggctgcactacagcggaagcatcaacgcctggagcaccaaggagccattcagctggatcaaagtggatctgctggccccaatgatcatccacggaatcaagacccagggagcccggcagaagttcagcagcctgtacatcagccagttcatcatcatgtacagcctggatggaaagaagtggcagacctaccggggaaacagcaccggaaccctgatggtgttcttcggaaacgtggatagcagcggaatcaagcacaacatcttcaacccaccaatcatcgcccgatacatccggctgcacccaacccactacagcatcagaagcaccctgcggatggagctgatgggatgtgatctgaacagctgctccatgccactgggaatggagagcaaggccatcagcgatgcccagatcaccgccagcagctacttcaccaacatgttcgccacctggagcccaagcaaggcccggctgcacctgcagggacggagcaacgcctggcggccacaggtgaataacccaaaggagtggctgcaggtggatttccagaagaccatgaaggtgaccggagtgaccacccagggagtgaagagcctgctgactagcatgtatgtgaaggagttcctgatcagcagcagccaggatggacaccagtggaccctgttcttccagaacggaaaggtgaaggtgttccagggaaaccaggatagcttcaccccagtggtgaacagcctggatccaccactgctgacccgatacctgcggatccacccacagagctgggtgcaccagatcgccctgagaatggaggtgctgggatgcgaggcccaggatctgtactgatgagcatgcaataaagtctgagtgggcggcagcctgtgtgtgcctgggttctctctgtcccggaatgtgcaaacaatggaggtgctcgagtagataagtagcatggcgggttaatcattaactacaaggaacccctagtgatggagttggccactccctctctgcgcgctcgctcgctcactgaggccgggcgaccaaaggtcgcccgacgcccgggctttgcccgggcggcctcagtgagcgagcgagcgcgcagccttaattaacctaattcactggccgtcgttttacaacgtcgtgactgggaaaaccctggcgttacccaacttaatcgccttgcagcacatccccctttcgccagctggcgtaatagcgaagaggcccgcaccgatcgcccttcccaacagttgcgcagcctgaatggcgaatgggacgcgccctgtagcggcgcattaagcgcggcgggtgtggtggttacgcgcagcgtgaccgctacacttgccagcgccctagcgcccgctcctttcgctttcttcccttcctttctcgccacgttcgccggctttccccgtcaagctctaaatcgggggctccctttagggttccgatttagtgctttacggcacctcgaccccaaaaaacttgattagggtgatggttcacgtagtgggccatcgccctgatagacggtttttcgccctttgacgttggagtccacgttctttaatagtggactcttgttccaaactggaacaacactcaaccctatctcggtctattcttttgatttataagggattttgccgatttcggcctattggttaaaaaatgagctgatttaacaaaaatttaacgcgaattttaacaaaatattaacgcttacaatttaggtggcacttttcggggaaatgtgcgcggaacccctatttgtttatttttctaaatacattcaaatatgtatccgctcatgagacaataaccctgataaatgcttcaataatattgaaaaaggaagagtatgagtattcaacatttccgtgtcgcccttattcccttttttgcggcattttgccttcctgtttttgctcacccagaaacgctggtgaaagtaaaagatgctgaagatcagttgggtgcacgagtgggttacatcgaactggatctcaacagcggtaagatccttgagagttttcgccccgaagaacgttttccaatgatgagcacttttaaagttctgctatgtggcgcggtattatcccgtattgacgccgggcaagagcaactcggtcgccgcatacactattctcagaatgacttggttgagtactcaccagtcacagaaaagcatcttacggatggcatgacagtaagagaattatgcagtgctgccataaccatgagtgataacactgcggccaacttacttctgacaacgatcggaggaccgaaggagctaaccgcttttttgcacaacatgggggatcatgtaactcgccttgatcgttgggaaccggagctgaatgaagccataccaaacgacgagcgtgacaccacgatgcctgtagcaatggcaacaacgttgcgcaaactattaactggcgaactacttactctagcttcccggcaacaattaatagactggatggaggcggataaagttgcaggaccacttctgcgctcggcccttccggctggctggtttattgctgataaatctggagccggtgagcgtgggtctcgcggtatcattgcagcactggggccagatggtaagccctcccgtatcgtagttatctacacgacggggagtcaggcaactatggatgaacgaaatagacagatcgctgagataggtgcctcactgattaagcattggtaactgtcagaccaagtttactcatatatactttagattgatttaaaacttcatttttaatttaaaaggatctaggtgaagatcctttttgataatctcatgaccaaaatcccttaacgtgagttttcgttccactgagcgtcagaccccgtagaaaagatcaaaggatcttcttgagatcctttttttctgcgcgtaatctgctgcttgcaaacaaaaaaaccaccgctaccagcggtggtttgtttgccggatcaagagctaccaactctttttccgaaggtaactggcttcagcagagcgcagataccaaatactgttcttctagtgtagccgtagttaggccaccacttcaagaactctgtagcaccgcctacatacctcgctctgctaatcctgttaccagtggctgctgccagtggcgataagtcgtgtcttaccgggttggactcaagacgatagttaccggataaggcgcagcggtcgggctgaacggggggttcgtgcacacagcccagcttggagcgaacgacctacaccgaactgagatacctacagcgtgagctatgagaaagcgccacgcttcccgaagggagaaaggcggacaggtatccggtaagcggcagggtcggaacaggagagcgcacgagggagcttccagggggaaacgcctggtatctttatagtcctgtcgggtttcgccacctctgacttgagcgtcgatttttgtgatgctcgtcaggggggcggagcctatggaaaaacgccagcaacgcggcctttttacggttcctggccttttgctggccttttgctcacatgttctttcctgcgttatcccctgattctgtggataaccgtattaccgcctttgagtgagctgataccgctcgccgcagccgaacgaccgagcgcagcgagtcagtgagcgaggaagcggaagagcgcccaatacgcaaaccgcctctccccgcgcgttggccgattcattaatgcagctggcacgacaggtttcccgactggaaagcgggcagtgagcgcaacgcaattaatgtgagttagctcactcattaggcaccccaggctttacactttatgcttccggctcgtatgttgtgtggaattgtgagcggataacaatttcacacaggaaacagctatgaccatgattacgccagatttaattaagg

SEQ ID NO: 15 - DNA, 7948 bp, Artificial Sequence
  constructed sequence
ctgcgcgctcgctcgctcactgaggccgcccgggcaaagcccgggcgtcgggcgacctttggtcgcccggcctcagtgagcgagcgagcgcgcagagagggagtggccaactccatcactaggggttccttgtagttaatgattaacccgccatgctacttatctacttaagctacctcgtgatcgcccggcccctgttcaaacatgtcctaatactctgtctctgcaagggtcatcagtagttttccatcttactcaacatcctcccagtggaattctggacacaggacgctgtggtttctgagccagggggcgactcagatcccagccagtggacttagcccctgtttgctcctccgataactggggtgaccttggttaatattcaccagcagcctcccccgttgcccctctggatccactgcttaaatacggacgaggacagggccctgtctcctcagcttcaggcaccaccactgacctgggacagtgaatagcggccgccaccatgcagatcgagctgagcacctgcttcttcctgtgcctgctgcggttctgcttctccgccacccggcggtactacctgggagccgtggagctgagctgggattacatgcagagcgatctgggagagctgccagtggatgcccggttcccaccacgggtgccaaagagcttcccattcaacaccagcgtggtgtacaagaagaccctgttcgtggagttcaccgatcacctgttcaacatcgccaagccacggccaccctggatgggactgctgggaccaaccatccaggccgaggtgtacgataccgtggtgatcaccctgaagaacatggcctctcatcctgtgtccctgcacgccgtgggagtgagctactggaaggccagcgagggagccgagtacgatgatcagaccagccagcgggagaaggaggatgataaggtgttcccaggaggaagccacacctacgtgtggcaggtgctgaaggagaacggaccaatggccagcgatccactgtgcctgacctacagctacctgagccacgtggatctggtgaaggatctgaacagcggactgatcggagccctgctggtgtgccgggagggaagcctggccaaggagaagacccagaccctgcacaagttcatcctgctgttcgccgtgttcgatgagggaaagagctggcacagcgagaccaagaacagcctgatgcaggatcgggatgccgccagcgcccgggcctggccaaagatgcacaccgtgaacggatacgtgaaccggagcctgccaggactgatcggatgccaccggaagagcgtgtactggcacgtgatcggaatgggaaccaccccagaggtgcactctatcttcctggagggacacacctttctggtgcggaaccaccggcaggccagcctggagatcagcccaatcaccttcctgaccgcccagaccctgctgatggatctgggacagttcctgctgttctgccatatcagcagccaccagcacgatggaatggaggcctacgtgaaggtggatagctgcccagaggagccacagctgcggatgaagaacaacgaggaggccgaggattacgatgatgatctgaccgatagcgagatggatgtggtgcggttcgatgatgataacagcccaagcttcatccagatccggagcgtggccaagaagcacccaaagacctgggtgcactacatcgccgccgaggaggaggattgggattacgccccactggtgctggcccctgatgatcggagctacaagagccagtacctgaacaacggaccacagcggatcggacggaagtacaaaaaagtgcggttcatggcctacaccgatgagaccttcaagacccgggaggccatccagcacgagagcggaatcctgggaccactgctgtacggagaggtgggagataccctgctgatcatcttcaagaaccaggccagccggccatacaacatctacccacacggaatcaccgatgtgcggccactgtacagccggcggctgccaaagggagtgaagcacctgaaggatttcccaatcctgccaggagagatcttcaagtacaagtggacagtgacagtggaggatggaccaaccaagtctgatccaagatgcctgaccagatactacagcagctttgtgaacatggagagagacctggcctctggactgattggaccactgctgatctgctacaaggagtctgtggatcagagaggaaaccagatcatgtctgataagagaaatgtgatcctgttctctgtgtttgatgagaacagaagctggtacctgacagagaacatccagagattcctgccaaacccagccggagtgcagctggaggatccagagttccaggccagcaacatcatgcacagcatcaacggatacgtgttcgatagcctgcagctgagcgtgtgcctgcacgaggtggcctattggtatatcctgagcatcggagcccagaccgatttcctgagcgtgttcttcagcggatacaccttcaagcacaagatggtgtacgaggataccctgaccctgttcccattctccggagagaccgtgttcatgagcatggagaacccaggactgtggatcctgggatgccacaactctgatttcagaaacagaggaatgactgccctgctgaaagtgtccagctgtgataagaacactggagattactatgaggatagctatgaggatatctctgcctacctgctgagcaagaacaatgccattgagccaagaagcttcagccagaacccaccagtgctgaagagacaccagagagagatcaccagaaccaccctgcagtctgatcaggaggagattgattatgatgataccatctctgtggagatgaagaaggaggattttgatatctatgatgaggatgagaaccagagcccaagaagcttccagaagaagaccagacactacttcatcgctgcagtggagagactgtgggattatggaatgagcagcagcccacacgtgctgagaaacagagcccagagcggatctgtgccacagttcaagaaggtggtgttccaggagttcaccgatggaagcttcacccagccactgtaccggggagagctgaacgagcacctgggactgctgggaccatacatccgggccgaggtggaggataacatcatggtgaccttccggaaccaggccagccggccatacagcttctacagcagcctgatcagctacgaggaggatcagcggcagggagccgagccacggaagaacttcgtgaagccaaacgagaccaagacctacttctggaaggtgcagcaccacatggccccaaccaaggatgagttcgattgcaaggcctgggcctacttcagcgatgtggatctggagaaggatgtgcacagcggactgatcggaccactgctggtgtgccacaccaacaccctgaacccagcccacggacggcaggtgaccgtgcaggagttcgccctgttcttcaccatcttcgatgagaccaagagctggtacttcaccgagaacatggagcggaactgccgggccccttgcaacatccagatggaggatccaaccttcaaggagaactaccggttccacgccatcaacggatacatcatggataccctgccaggactggtgatggcccaggatcagcggatccggtggtacctgctgagcatgggaagcaacgagaacatccacagcatccacttcagcggacacgtgttcaccgtgcggaagaaggaggagtacaagatggccctgtacaacctgtacccaggagtgttcgagaccgtggagatgctgccaagcaaggccggaatctggcgggtggagtgcctgatcggagagcacctgcacgccggaatgagcaccctgttcctggtgtacagcaacaagtgccagaccccactgggaatggccagcggacacatccgggatttccagatcaccgccagcggacagtacggacagtgggccccaaagctggcccggctgcactacagcggaagcatcaacgcctggagcaccaaggagccattcagctggatcaaagtggatctgctggccccaatgatcatccacggaatcaagacccagggagcccggcagaagttcagcagcctgtacatcagccagttcatcatcatgtacagcctggatggaaagaagtggcagacctaccggggaaacagcaccggaaccctgatggtgttcttcggaaacgtggatagcagcggaatcaagcacaacatcttcaacccaccaatcatcgcccgatacatccggctgcacccaacccactacagcatcagaagcaccctgcggatggagctgatgggatgtgatctgaacagctgctccatgccactgggaatggagagcaaggccatcagcgatgcccagatcaccgccagcagctacttcaccaacatgttcgccacctggagcccaagcaaggcccggctgcacctgcagggacggagcaacgcctggcggccacaggtgaataacccaaaggagtggctgcaggtggatttccagaagaccatgaaggtgaccggagtgaccacccagggagtgaagagcctgctgactagcatgtatgtgaaggagttcctgatcagcagcagccaggatggacaccagtggaccctgttcttccagaacggaaaggtgaaggtgttccagggaaaccaggatagcttcaccccagtggtgaacagcctggatccaccactgctgacccgatacctgcggatccacccacagagctgggtgcaccagatcgccctgagaatggaggtgctgggatgcgaggcccaggatctgtactgatgagcatgcaataaagtctgagtgggcggcagcctgtgtgtgcctgggttctctctgtcccggaatgtgcaaacaatggaggtgctcgagtagataagtagcatggcgggttaatcattaactacaaggaacccctagtgatggagttggccactccctctctgcgcgctcgctcgctcactgaggccgggcgaccaaaggtcgcccgacgcccgggctttgcccgggcggcctcagtgagcgagcgagcgcgcagccttaattaacctaattcactggccgtcgttttacaacgtcgtgactgggaaaaccctggcgttacccaacttaatcgccttgcagcacatccccctttcgccagctggcgtaatagcgaagaggcccgcaccgatcgcccttcccaacagttgcgcagcctgaatggcgaatgggacgcgccctgtagcggcgcattaagcgcggcgggtgtggtggttacgcgcagcgtgaccgctacacttgccagcgccctagcgcccgctcctttcgctttcttcccttcctttctcgccacgttcgccggctttccccgtcaagctctaaatcgggggctccctttagggttccgatttagtgctttacggcacctcgaccccaaaaaacttgattagggtgatggttcacgtagtgggccatcgccctgatagacggtttttcgccctttgacgttggagtccacgttctttaatagtggactcttgttccaaactggaacaacactcaaccctatctcggtctattcttttgatttataagggattttgccgatttcggcctattggttaaaaaatgagctgatttaacaaaaatttaacgcgaattttaacaaaatattaacgcttacaatttaggtggcacttttcggggaaatgtgcgcggaacccctatttgtttatttttctaaatacattcaaatatgtatccgctcatgagacaataaccctgataaatgcttcaataatattgaaaaaggaagagtatgagtattcaacatttccgtgtcgcccttattcccttttttgcggcattttgccttcctgtttttgctcacccagaaacgctggtgaaagtaaaagatgctgaagatcagttgggtgcacgagtgggttacatcgaactggatctcaacagcggtaagatccttgagagttttcgccccgaagaacgttttccaatgatgagcacttttaaagttctgctatgtggcgcggtattatcccgtattgacgccgggcaagagcaactcggtcgccgcatacactattctcagaatgacttggttgagtactcaccagtcacagaaaagcatcttacggatggcatgacagtaagagaattatgcagtgctgccataaccatgagtgataacactgcggccaacttacttctgacaacgatcggaggaccgaaggagctaaccgcttttttgcacaacatgggggatcatgtaactcgccttgatcgttgggaaccggagctgaatgaagccataccaaacgacgagcgtgacaccacgatgcctgtagcaatggcaacaacgttgcgcaaactattaactggcgaactacttactctagcttcccggcaacaattaatagactggatggaggcggataaagttgcaggaccacttctgcgctcggcccttccggctggctggtttattgctgataaatctggagccggtgagcgtgggtctcgcggtatcattgcagcactggggccagatggtaagccctcccgtatcgtagttatctacacgacggggagtcaggcaactatggatgaacgaaatagacagatcgctgagataggtgcctcactgattaagcattggtaactgtcagaccaagtttactcatatatactttagattgatttaaaacttcatttttaatttaaaaggatctaggtgaagatcctttttgataatctcatgaccaaaatcccttaacgtgagttttcgttccactgagcgtcagaccccgtagaaaagatcaaaggatcttcttgagatcctttttttctgcgcgtaatctgctgcttgcaaacaaaaaaaccaccgctaccagcggtggtttgtttgccggatcaagagctaccaactctttttccgaaggtaactggcttcagcagagcgcagataccaaatactgttcttctagtgtagccgtagttaggccaccacttcaagaactctgtagcaccgcctacatacctcgctctgctaatcctgttaccagtggctgctgccagtggcgataagtcgtgtcttaccgggttggactcaagacgatagttaccggataaggcgcagcggtcgggctgaacggggggttcgtgcacacagcccagcttggagcgaacgacctacaccgaactgagatacctacagcgtgagctatgagaaagcgccacgcttcccgaagggagaaaggcggacaggtatccggtaagcggcagggtcggaacaggagagcgcacgagggagcttccagggggaaacgcctggtatctttatagtcctgtcgggtttcgccacctctgacttgagcgtcgatttttgtgatgctcgtcaggggggcggagcctatggaaaaacgccagcaacgcggcctttttacggttcctggccttttgctggccttttgctcacatgttctttcctgcgttatcccctgattctgtggataaccgtattaccgcctttgagtgagctgataccgctcgccgcagccgaacgaccgagcgcagcgagtcagtgagcgaggaagcggaagagcgcccaatacgcaaaccgcctctccccgcgcgttggccgattcattaatgcagctggcacgacaggtttcccgactggaaagcgggcagtgagcgcaacgcaattaatgtgagttagctcactcattaggcaccccaggctttacactttatgcttccggctcgtatgttgtgtggaattgtgagcggataacaatttcacacaggaaacagctatgaccatgattacgccagatttaattaagg

SEQ ID NO: 16 - DNA, 8032 bp, Artificial Sequence
  constructed sequence
ctgcgcgctcgctcgctcactgaggccgcccgggcaaagcccgggcgtcgggcgacctttggtcgcccggcctcagtgagcgagcgagcgcgcagagagggagtggccaactccatcactaggggttccttgtagttaatgattaacccgccatgctacttatctacttaagctacctcgtgatcgcccggcccctgttcaaacatgtcctaatactctgtctctgcaagggtcatcagtagttttccatcttactcaacatcctcccagtgaggttaatttttaaactgtttgctctggttaataatctcaggaggttaatttttaaactgtttgctctggttaataatctcagggaattctggacacaggacgctgtggtttctgagccagggggcgactcagatcccagccagtggacttagcccctgtttgctcctccgataactggggtgaccttggttaatattcaccagcagcctcccccgttgcccctctggatccactgcttaaatacggacgaggacagggccctgtctcctcagcttcaggcaccaccactgacctgggacagtgaatagcggccgccaccatgcagatcgagctgagcacctgcttcttcctgtgcctgctgcggttctgcttctccgccacccggcggtactacctgggagccgtggagctgagctgggattacatgcagagcgatctgggagagctgccagtggatgcccggttcccaccacgggtgccaaagagcttcccattcaacaccagcgtggtgtacaagaagaccctgttcgtggagttcaccgatcacctgttcaacatcgccaagccacggccaccctggatgggactgctgggaccaaccatccaggccgaggtgtacgataccgtggtgatcaccctgaagaacatggcctctcatcctgtgtccctgcacgccgtgggagtgagctactggaaggccagcgagggagccgagtacgatgatcagaccagccagcgggagaaggaggatgataaggtgttcccaggaggaagccacacctacgtgtggcaggtgctgaaggagaacggaccaatggccagcgatccactgtgcctgacctacagctacctgagccacgtggatctggtgaaggatctgaacagcggactgatcggagccctgctggtgtgccgggagggaagcctggccaaggagaagacccagaccctgcacaagttcatcctgctgttcgccgtgttcgatgagggaaagagctggcacagcgagaccaagaacagcctgatgcaggatcgggatgccgccagcgcccgggcctggccaaagatgcacaccgtgaacggatacgtgaaccggagcctgccaggactgatcggatgccaccggaagagcgtgtactggcacgtgatcggaatgggaaccaccccagaggtgcactctatcttcctggagggacacacctttctggtgcggaaccaccggcaggccagcctggagatcagcccaatcaccttcctgaccgcccagaccctgctgatggatctgggacagttcctgctgttctgccatatcagcagccaccagcacgatggaatggaggcctacgtgaaggtggatagctgcccagaggagccacagctgcggatgaagaacaacgaggaggccgaggattacgatgatgatctgaccgatagcgagatggatgtggtgcggttcgatgatgataacagcccaagcttcatccagatccggagcgtggccaagaagcacccaaagacctgggtgcactacatcgccgccgaggaggaggattgggattacgccccactggtgctggcccctgatgatcggagctacaagagccagtacctgaacaacggaccacagcggatcggacggaagtacaaaaaagtgcggttcatggcctacaccgatgagaccttcaagacccgggaggccatccagcacgagagcggaatcctgggaccactgctgtacggagaggtgggagataccctgctgatcatcttcaagaaccaggccagccggccatacaacatctacccacacggaatcaccgatgtgcggccactgtacagccggcggctgccaaagggagtgaagcacctgaaggatttcccaatcctgccaggagagatcttcaagtacaagtggacagtgacagtggaggatggaccaaccaagtctgatccaagatgcctgaccagatactacagcagctttgtgaacatggagagagacctggcctctggactgattggaccactgctgatctgctacaaggagtctgtggatcagagaggaaaccagatcatgtctgataagagaaatgtgatcctgttctctgtgtttgatgagaacagaagctggtacctgacagagaacatccagagattcctgccaaacccagccggagtgcagctggaggatccagagttccaggccagcaacatcatgcacagcatcaacggatacgtgttcgatagcctgcagctgagcgtgtgcctgcacgaggtggcctattggtatatcctgagcatcggagcccagaccgatttcctgagcgtgttcttcagcggatacaccttcaagcacaagatggtgtacgaggataccctgaccctgttcccattctccggagagaccgtgttcatgagcatggagaacccaggactgtggatcctgggatgccacaactctgatttcagaaacagaggaatgactgccctgctgaaagtgtccagctgtgataagaacactggagattactatgaggatagctatgaggatatctctgcctacctgctgagcaagaacaatgccattgagccaagaagcttcagccagaacccaccagtgctgaagagacaccagagagagatcaccagaaccaccctgcagtctgatcaggaggagattgattatgatgataccatctctgtggagatgaagaaggaggattttgatatctatgatgaggatgagaaccagagcccaagaagcttccagaagaagaccagacactacttcatcgctgcagtggagagactgtgggattatggaatgagcagcagcccacacgtgctgagaaacagagcccagagcggatctgtgccacagttcaagaaggtggtgttccaggagttcaccgatggaagcttcacccagccactgtaccggggagagctgaacgagcacctgggactgctgggaccatacatccgggccgaggtggaggataacatcatggtgaccttccggaaccaggccagccggccatacagcttctacagcagcctgatcagctacgaggaggatcagcggcagggagccgagccacggaagaacttcgtgaagccaaacgagaccaagacctacttctggaaggtgcagcaccacatggccccaaccaaggatgagttcgattgcaaggcctgggcctacttcagcgatgtggatctggagaaggatgtgcacagcggactgatcggaccactgctggtgtgccacaccaacaccctgaacccagcccacggacggcaggtgaccgtgcaggagttcgccctgttcttcaccatcttcgatgagaccaagagctggtacttcaccgagaacatggagcggaactgccgggccccttgcaacatccagatggaggatccaaccttcaaggagaactaccggttccacgccatcaacggatacatcatggataccctgccaggactggtgatggcccaggatcagcggatccggtggtacctgctgagcatgggaagcaacgagaacatccacagcatccacttcagcggacacgtgttcaccgtgcggaagaaggaggagtacaagatggccctgtacaacctgtacccaggagtgttcgagaccgtggagatgctgccaagcaaggccggaatctggcgggtggagtgcctgatcggagagcacctgcacgccggaatgagcaccctgttcctggtgtacagcaacaagtgccagaccccactgggaatggccagcggacacatccgggatttccagatcaccgccagcggacagtacggacagtgggccccaaagctggcccggctgcactacagcggaagcatcaacgcctggagcaccaaggagccattcagctggatcaaagtggatctgctggccccaatgatcatccacggaatcaagacccagggagcccggcagaagttcagcagcctgtacatcagccagttcatcatcatgtacagcctggatggaaagaagtggcagacctaccggggaaacagcaccggaaccctgatggtgttcttcggaaacgtggatagcagcggaatcaagcacaacatcttcaacccaccaatcatcgcccgatacatccggctgcacccaacccactacagcatcagaagcaccctgcggatggagctgatgggatgtgatctgaacagctgctccatgccactgggaatggagagcaaggccatcagcgatgcccagatcaccgccagcagctacttcaccaacatgttcgccacctggagcccaagcaaggcccggctgcacctgcagggacggagcaacgcctggcggccacaggtgaataacccaaaggagtggctgcaggtggatttccagaagaccatgaaggtgaccggagtgaccacccagggagtgaagagcctgctgactagcatgtatgtgaaggagttcctgatcagcagcagccaggatggacaccagtggaccctgttcttccagaacggaaaggtgaaggtgttccagggaaaccaggatagcttcaccccagtggtgaacagcctggatccaccactgctgacccgatacctgcggatccacccacagagctgggtgcaccagatcgccctgagaatggaggtgctgggatgcgaggcccaggatctgtactgatgagcatgcaataaagtctgagtgggcggcagcctgtgtgtgcctgggttctctctgtcccggaatgtgcaaacaatggaggtgctcgagtagataagtagcatggcgggttaatcattaactacaaggaacccctagtgatggagttggccactccctctctgcgcgctcgctcgctcactgaggccgggcgaccaaaggtcgcccgacgcccgggctttgcccgggcggcctcagtgagcgagcgagcgcgcagccttaattaacctaattcactggccgtcgttttacaacgtcgtgactgggaaaaccctggcgttacccaacttaatcgccttgcagcacatccccctttcgccagctggcgtaatagcgaagaggcccgcaccgatcgcccttcccaacagttgcgcagcctgaatggcgaatgggacgcgccctgtagcggcgcattaagcgcggcgggtgtggtggttacgcgcagcgtgaccgctacacttgccagcgccctagcgcccgctcctttcgctttcttcccttcctttctcgccacgttcgccggctttccccgtcaagctctaaatcgggggctccctttagggttccgatttagtgctttacggcacctcgaccccaaaaaacttgattagggtgatggttcacgtagtgggccatcgccctgatagacggtttttcgccctttgacgttggagtccacgttctttaatagtggactcttgttccaaactggaacaacactcaaccctatctcggtctattcttttgatttataagggattttgccgatttcggcctattggttaaaaaatgagctgatttaacaaaaatttaacgcgaattttaacaaaatattaacgcttacaatttaggtggcacttttcggggaaatgtgcgcggaacccctatttgtttatttttctaaatacattcaaatatgtatccgctcatgagacaataaccctgataaatgcttcaataatattgaaaaaggaagagtatgagtattcaacatttccgtgtcgcccttattcccttttttgcggcattttgccttcctgtttttgctcacccagaaacgctggtgaaagtaaaagatgctgaagatcagttgggtgcacgagtgggttacatcgaactggatctcaacagcggtaagatccttgagagttttcgccccgaagaacgttttccaatgatgagcacttttaaagttctgctatgtggcgcggtattatcccgtattgacgccgggcaagagcaactcggtcgccgcatacactattctcagaatgacttggttgagtactcaccagtcacagaaaagcatcttacggatggcatgacagtaagagaattatgcagtgctgccataaccatgagtgataacactgcggccaacttacttctgacaacgatcggaggaccgaaggagctaaccgcttttttgcacaacatgggggatcatgtaactcgccttgatcgttgggaaccggagctgaatgaagccataccaaacgacgagcgtgacaccacgatgcctgtagcaatggcaacaacgttgcgcaaactattaactggcgaactacttactctagcttcccggcaacaattaatagactggatggaggcggataaagttgcaggaccacttctgcgctcggcccttccggctggctggtttattgctgataaatctggagccggtgagcgtgggtctcgcggtatcattgcagcactggggccagatggtaagccctcccgtatcgtagttatctacacgacggggagtcaggcaactatggatgaacgaaatagacagatcgctgagataggtgcctcactgattaagcattggtaactgtcagaccaagtttactcatatatactttagattgatttaaaacttcatttttaatttaaaaggatctaggtgaagatcctttttgataatctcatgaccaaaatcccttaacgtgagttttcgttccactgagcgtcagaccccgtagaaaagatcaaaggatcttcttgagatcctttttttctgcgcgtaatctgctgcttgcaaacaaaaaaaccaccgctaccagcggtggtttgtttgccggatcaagagctaccaactctttttccgaaggtaactggcttcagcagagcgcagataccaaatactgttcttctagtgtagccgtagttaggccaccacttcaagaactctgtagcaccgcctacatacctcgctctgctaatcctgttaccagtggctgctgccagtggcgataagtcgtgtcttaccgggttggactcaagacgatagttaccggataaggcgcagcggtcgggctgaacggggggttcgtgcacacagcccagcttggagcgaacgacctacaccgaactgagatacctacagcgtgagctatgagaaagcgccacgcttcccgaagggagaaaggcggacaggtatccggtaagcggcagggtcggaacaggagagcgcacgagggagcttccagggggaaacgcctggtatctttatagtcctgtcgggtttcgccacctctgacttgagcgtcgatttttgtgatgctcgtcaggggggcggagcctatggaaaaacgccagcaacgcggcctttttacggttcctggccttttgctggccttttgctcacatgttctttcctgcgttatcccctgattctgtggataaccgtattaccgcctttgagtgagctgataccgctcgccgcagccgaacgaccgagcgcagcgagtcagtgagcgaggaagcggaagagcgcccaatacgcaaaccgcctctccccgcgcgttggccgattcattaatgcagctggcacgacaggtttcccgactggaaagcgggcagtgagcgcaacgcaattaatgtgagttagctcactcattaggcaccccaggctttacactttatgcttccggctcgtatgttgtgtggaattgtgagcggataacaatttcacacaggaaacagctatgaccatgattacgccagatttaattaagg

SEQ ID NO: 17 - protein, 738 aa, Unknown
  AAVhu.37 capsid
MAADGYLPDWLEDNLSEGIREWWDLKPGAPKPKANQQKQDDGRGLVLPGYKYLGPFNGLDKGEPVNAADAAALEHDKAYDQQLKAGDNPYLRYNHADAEFQERLQEDTSFGGNLGRAVFQAKKRVLEPLGLVEEAAKTAPGKKRPVEPSPQRSPDSSTGIGKKGQQPAKKRLNFGQTGDSESVPDPQPIGEPPAGPSGLGSGTMAAGGGAPMADNNEGADGVGSSSGNWHCDSTWLGDRVITTSTRTWALPTYNNHLYKQISNGTSGGSTNDNTYFGYSTPWGYFDFNRFHCHFSPRDWQRLINNNWGFRPKRLSFKLFNIQVKEVTQNEGTKTIANNLTSTIQVFTDSEYQLPYVLGSAHQGCLPPFPADVFMIPQYGYLTLNNGSQAVGRSSFYCLEYFPSQMLRTGNNFEFSYTFEDVPFHSSYAHSQSLDRLMNPLIDQYLYYLSRTQSTGGTQGTQQLLFSQAGPANMSAQAKNWLPGPCYRQQRVSTTLSQNNNSNFAWTGATKYHLNGRDSLVNPGVAMATHKDDEERFFPSSGVLMFGKQGAGRDNVDYSSVMLTSEEEIKTTNPVATEQYGVVADNLQQTNTGPIVGNVNSQGALPGMVWQNRDVYLQGPIWAKIPHTDGNFHPSPLMGGFGLKHPPPQILIKNTPVPADPPTTFSQAKLASFITQYSTGQVSVEIEWELQKENSKRWNPEIQYTSNYYKSTNVDFAVNTEGTYSEPRPIGTRYLTRNL

SEQ ID NO: 18 - protein, 738 aa, Unknown
  AAVrh.10 capsid
MAADGYLPDWLEDNLSEGIREWWDLKPGAPKPKANQQKQDDGRGLVLPGYKYLGPFNGLDKGEPVNAADAAALEHDKAYDQQLKAGDNPYLRYNHADAEFQERLQEDTSFGGNLGRAVFQAKKRVLEPLGLVEEGAKTAPGKKRPVEPSPQRSPDSSTGIGKKGQQPAKKRLNFGQTGDSESVPDPQPIGEPPAGPSGLGSGTMAAGGGAPMADNNEGADGVGSSSGNWHCDSTWLGDRVITTSTRTWALPTYNNHLYKQISNGTSGGSTNDNTYFGYSTPWGYFDFNRFHCHFSPRDWQRLINNNWGFRPKRLNFKLFNIQVKEVTQNEGTKTIANNLTSTIQVFTDSEYQLPYVLGSAHQGCLPPFPADVFMIPQYGYLTLNNGSQAVGRSSFYCLEYFPSQMLRTGNNFEFSYQFEDVPFHSSYAHSQSLDRLMNPLIDQYLYYLSRTQSTGGTAGTQQLLFSQAGPNNMSAQAKNWLPGPCYRQQRVSTTLSQNNNSNFAWTGATKYHLNGRDSLVNPGVAMATHKDDEERFFPSSGVLMFGKQGAGKDNVDYSSVMLTSEEEIKTTNPVATEQYGVVADNLQQQNAAPIVGAVNSQGALPGMVWQNRDVYLQGPIWAKIPHTDGNFHPSPLMGGFGLKHPPPQILIKNTPVPADPPTTFSQAKLASFITQYSTGQVSVEIEWELQKENSKRWNPEIQYTSNYYKSTNVDFAVNTDGTYSEPRPIGTRYLTRNL

SEQ ID NO: 19 - DNA, 4371 bp, Artificial Sequence
  constructed sequence
atgcagatcgagctgtctacctgcttcttcctgtgcctgctgcggttctgcttcagcgccaccagacggtactatctgggcgccgtggaactgagctgggactacatgcagagcgacctgggcgagctgcccgtggacgccagattccctccaagagtgcccaagagcttccccttcaacacctccgtggtgtacaagaaaaccctgttcgtggaattcaccgaccacctgttcaatatcgccaagcccagacccccctggatgggcctgctgggacctacaattcaggccgaggtgtacgacaccgtcgtgatcaccctgaagaacatggccagccaccccgtgtctctgcacgccgtgggagtgtcctactggaaggcctctgagggcgccgagtacgacgatcagaccagccagcgcgagaaagaggacgacaaggtgttccctggcggcagccacacctacgtgtggcaggtgctgaaagaaaacggccccatggcctccgaccctctgtgcctgacatacagctacctgagccacgtggacctcgtgaaggacctgaacagcggcctgatcggagccctgctcgtgtgtagagagggcagcctggccaaagagaaaacccagaccctgcacaagttcatcctgctgttcgccgtgttcgacgagggcaagagctggcacagcgagacaaagaacagcctgatgcaggaccgggacgccgcctctgctagagcctggcccaaaatgcacaccgtgaacggctacgtgaacagaagcctgcccggactgatcggctgccaccggaagtctgtgtactggcacgtgatcggcatgggcaccacccctgaggtgcacagcatctttctggaaggacacacctttctcgtgcggaaccaccggcaggccagcctggaaatcagccctatcaccttcctgaccgcccagacactgctgatggacctgggccagtttctgctgttctgccacatcagctcccaccagcacgacggcatggaagcctacgtgaaggtggacagctgccccgaggaaccccagctgcggatgaagaacaacgaggaagccgaggactacgacgacgacctgaccgacagcgagatggacgtggtgcgcttcgacgacgataacagccccagcttcatccagatcagaagcgtggccaagaagcaccccaagacctgggtgcactatatcgccgccgaggaagaggactgggattacgcccctctggtgctggcccccgacgacagaagctacaagagccagtacctgaacaacggcccccagcggatcggccggaagtataagaaagtgcggttcatggcctacaccgacgagacattcaagaccagagaggccatccagcacgagagcggcatcctgggccctctgctgtatggcgaagtgggcgacaccctgctgatcatcttcaagaaccaggccagcagaccctacaacatctaccctcacggcatcaccgacgtgcggcccctgtactctagaaggctgcccaagggcgtgaaacacctgaaggacttccccatcctgcccggcgagatcttcaagtacaagtggaccgtgaccgtggaagatggccccaccaagagcgaccccagatgcctgacacggtactatagcagcttcgtgaacatggaacgggacctggcctccggcctgattggcccactgctgatctgctacaaagaaagcgtggaccagcggggcaaccagatcatgagcgacaagcggaacgtgatcctgtttagcgtgttcgatgagaaccggtcctggtatctgaccgagaatatccagcggttcctgcccaaccctgccggcgtgcagctggaagatcctgagttccaggcctccaacatcatgcactccatcaatggctatgtgttcgacagcctgcagctgagcgtgtgcctgcacgaggtggcctactggtacatcctgagcatcggggcccagaccgacttcctgtccgtgttcttctccggctacaccttcaagcacaagatggtgtacgaggataccctgaccctgttcccctttagcggcgaaaccgtgttcatgagcatggaaaaccccggcctgtggatcctgggctgccacaacagcgacttccggaacagaggcatgaccgccctgctgaaggtgtccagctgcgacaagaacaccggcgactactacgaggacagctatgaggacatcagcgcctacctgctgagcaagaacaacgccatcgagcccagaagcttcagccagaacccccccgtgctgaagcggcaccagagagagatcacccggaccaccctgcagtccgaccaggaagagatcgattacgacgacaccatcagcgtggaaatgaagaaagaagatttcgacatctacgacgaggacgagaaccagagcccccggtcctttcagaaaaagacccggcactacttcattgccgctgtggaacggctgtgggactacggcatgagcagcagccctcacgtgctgagaaacagggcccagagcggcagcgtgccccagttcaagaaagtggtgttccaggaattcacagacggcagcttcacccagcctctgtaccgcggcgagctgaacgagcacctgggactgctgggcccctatatcagagccgaagtggaagataacatcatggtcaccttccggaatcaggcctcccggccctacagcttctacagctccctgatcagctacgaagaggaccagagacagggcgctgagccccggaagaacttcgtgaagcccaacgagactaagacctacttttggaaggtgcagcaccacatggcccctacaaaggacgagttcgactgcaaggcctgggcctacttctccgacgtggacctggaaaaggacgtgcactctgggctgatcggccccctgctcgtgtgccacaccaacaccctgaatcccgcccacggcagacaggtgacagtgcaggaattcgccctgttcttcaccatcttcgacgaaacaaagagctggtacttcaccgaaaacatggaaagaaactgccgggctccctgcaacatccagatggaagatcccaccttcaaagagaactaccggttccacgccatcaacggctacatcatggacacactgcccggcctcgtgatggctcaggatcagcggatccggtggtatctgctgtccatgggctccaacgagaacatccacagcatccacttcagcggccacgtgttcaccgtgcggaaaaaagaagagtacaaaatggccctgtacaacctgtaccctggggtgttcgagacagtggaaatgctgcccagcaaggccggcatctggcgggtggagtgtctgatcggcgagcacctgcacgctgggatgagcacactgtttctggtgtacagcaacaagtgccagacacctctgggcatggcctctggccacatccgggactttcagatcacagccagcggccagtacggccagtgggccccaaaactggccagactgcactacagcggcagcatcaacgcctggtccaccaaagagcccttcagctggatcaaggtggacctgctggctcccatgatcatccacggaatcaagacccagggcgccagacagaagttcagcagcctgtacatcagccagttcatcatcatgtacagcctggacggcaagaagtggcagacctaccggggcaatagcaccggcaccctgatggtgttcttcggcaacgtggactccagcggcattaagcacaacatcttcaacccccccatcattgcccggtacatccggctgcaccccacccactacagcatccggtccaccctgagaatggaactgatgggctgcgacctgaactcctgctccatgcccctggggatggaaagcaaggccatctccgacgcccagatcaccgcctccagctacttcaccaacatgttcgccacctggtccccatccaaggcccggctgcacctgcagggcagaagcaatgcttggaggcctcaggtgaacaaccccaaagagtggctgcaggtggacttccagaaaaccatgaaagtgaccggcgtgaccacccagggcgtgaagtctctgctgacctctatgtacgtgaaagagttcctgatctccagcagccaggacggccaccagtggaccctgtttttccagaacggcaaagtgaaagtgtttcaggggaaccaggactccttcacccccgtcgtgaatagcctggaccctccactgctgaccagatacctgcggatccaccctcagagttgggtgcaccagattgctctgcggatggaagtgctgggatgcgaggcccaggacctgtac

SEQ ID NO: 20 - protein, 736 aa, Unknown
  AAV3B capsid
MAADGYLPDWLEDNLSEGIREWWALKPGVPQPKANQQHQDNRRGLVLPGYKYLGPGNGLDKGEPVNEADAAALEHDKAYDQQLKAGDNPYLKYNHADAEFQERLQEDTSFGGNLGRAVFQAKKRILEPLGLVEEAAKTAPGKKRPVDQSPQEPDSSSGVGKSGKQPARKRLNFGQTGDSESVPDPQPLGEPPAAPTSLGSNTMASGGGAPMADNNEGADGVGNSSGNWHCDSQWLGDRVITTSTRTWALPTYNNHLYKQISSQSGASNDNHYFGYSTPWGYFDFNRFHCHFSPRDWQRLINNNWGFRPKKLSFKLFNIQVKEVTQNDGTTTIANNLTSTVQVFTDSEYQLPYVLGSAHQGCLPPFPADVFMVPQYGYLTLNNGSQAVGRSSFYCLEYFPSQMLRTGNNFQFSYTFEDVPFHSSYAHSQSLDRLMNPLIDQYLYYLNRTQGTTSGTTNQSRLLFSQAGPQSMSLQARNWLPGPCYRQQRLSKTANDNNNSNFPWTAASKYHLNGRDSLVNPGPAMASHKDDEEKFFPMHGNLIFGKEGTTASNAELDNVMITDEEEIRTTNPVATEQYGTVANNLQSSNTAPTTRTVNDQGALPGMVWQDRDVYLQGPIWAKIPHTDGHFHPSPLMGGFGLKHPPPQIMIKNTPVPANPPTTFSPAKFASFITQYSTGQVSVEIEWELQKENSKRWNPEIQYTSNYNKSVNVDFTVDTNGVYSEPRPIGTRYLTRNL